European Patent Specification EP 4 007 636 B1, published June 19, 2024. Title: COMPOSITIONS COMPRISING BOVINE ADRENAL MEDULLA 8-22 (BAM8-22) PEPTIDE ANALOGS AND METHODS OF USE. Applicant: OKYO Pharma Limited. The sequence listing filed with the application follows.

SEQUENCE LISTING (54 sequences)

SEQ ID NO: 1 - protein, 13 aa, Artificial Sequence
  artificial peptide composition
  MISC_FEATURE (1)..(1): Xaa at position 1 is glycine or D-glycine
  MISC_FEATURE (2)..(2): Xaa at position 2 is arginine, D-arginine, norarginine, asparagine, D-asparagine, pyroglutamic acid (PyroG), or 4-guanidino butyric acid (Gba)
  MISC_FEATURE (3)..(3): Xaa at position 3 is proline or D-proline
  MISC_FEATURE (4)..(4): Xaa at position 4 is glutamic acid or aspartic acid
  MISC_FEATURE (7)..(7): Xaa at position 7 is methionine or alanine
  MISC_FEATURE (8)..(8): Xaa at position 8 is glutamic acid or aspartic acid
  MISC_FEATURE (9)..(9): Xaa at position 9 is tyrosine, phenylalanine, tryptophan, or 4-pyridyl alanine
  MISC_FEATURE (10)..(10): Xaa at position 10 is glutamine or asparagine
  MISC_FEATURE (13)..(13): Xaa at position 13 is tyrosine, D-tyrosine, serine, or D-serine
XXXXWWXXXXKRX

SEQ ID NO: 2 - protein, 13 aa, Artificial Sequence
  artificial peptide composition
  MISC_FEATURE (1)..(1): Xaa at position 1 is glycine or D-glycine
  MISC_FEATURE (13)..(13): Xaa at position 13 is tyrosine or D-tyrosine
XRPEWWMDYQKRX

SEQ ID NO: 3 - protein, 13 aa, Artificial Sequence
  artificial peptide composition
GRPEWWMDYQKRY

SEQ ID NO: 4 - protein, 13 aa, Artificial Sequence
  artificial peptide composition
  MISC_FEATURE (1)..(1): Xaa at position 1 is D-glycine
  MISC_FEATURE (13)..(13): Xaa at position 13 is D-tyrosine
XRPEWWMDYQKRX

SEQ ID NO: 5 - protein, 12 aa, Artificial Sequence
  artificial peptide composition
  MISC_FEATURE (1)..(1): Xaa at position 1 is arginine, D-arginine, norarginine, asparagine, D-asparagine, aspartic acid, D-aspartic acid, pyroglutamic acid (PyroG), or 4-guanidino butyric acid (Gba)
  MISC_FEATURE (3)..(3): Xaa at position 3 is glutamic acid or aspartic acid
  MISC_FEATURE (6)..(6): Xaa at position 6 is methionine or alanine
  MISC_FEATURE (7)..(7): Xaa at position 7 is glutamic acid or aspartic acid
  MISC_FEATURE (8)..(8): Xaa at position 8 is tyrosine, phenylalanine, tryptophan, or 4-pyridyl alanine (4-Pal)
  MISC_FEATURE (9)..(9): Xaa at position 9 is glutamine or asparagine
  MISC_FEATURE (12)..(12): Xaa at position 12 is tyrosine, D-tyrosine, serine, or D-serine
XPXWWXXXXKRX

SEQ ID NO: 6 - protein, 12 aa, Artificial Sequence
  artificial peptide composition
RPEWWMDYQKRY

SEQ ID NO: 7 - protein, 12 aa, Artificial Sequence
  artificial peptide composition
  MISC_FEATURE (1)..(1): Xaa at position 1 is D-asparagine
  MISC_FEATURE (12)..(12): Xaa at position 12 is D-tyrosine
XPEWWMDYQKRX

SEQ ID NO: 8 - protein, 12 aa, Artificial Sequence
  artificial peptide sequence
  MISC_FEATURE (12)..(12): Xaa at position 12 is D-tyrosine
NPDWWMEYQKRX

SEQ ID NO: 9 - protein, 12 aa, Artificial Sequence
  artificial peptide composition
  MISC_FEATURE (12)..(12): Xaa at position 12 is D-serine
NPDWWMDFQKRX

SEQ ID NO: 10 - protein, 12 aa, Artificial Sequence
  artificial peptide composition
  MISC_FEATURE (1)..(1): Xaa at position 1 is pyroglutamic acid (PyroG)
  MISC_FEATURE (12)..(12): Xaa at position 12 is D-serine
XPDWWMEFNKRX

SEQ ID NO: 11 - protein, 12 aa, Artificial Sequence
  artificial peptide composition
  MISC_FEATURE (8)..(8): Xaa at position 8 is 4-pyridyl alanine (4-Pal)
  MISC_FEATURE (12)..(12): Xaa at position 12 is D-tyrosine
DPEWWMDXQKRX

SEQ ID NO: 12 - protein, 12 aa, Artificial Sequence
  artificial peptide composition
  MISC_FEATURE (1)..(1): Xaa at position 1 is 4-guanidino butyric acid (Gba)
  MISC_FEATURE (12)..(12): Xaa at position 12 is D-tyrosine
XPEWWMDYQKRX

SEQ ID NO: 13 - protein, 12 aa, Artificial Sequence
  artificial peptide composition
  MISC_FEATURE (1)..(1): Xaa at position 1 is 4-guanidino butyric acid (Gba)
  MISC_FEATURE (12)..(12): Xaa at position 12 is D-tyrosine
XPEWWMDWQKRX

SEQ ID NO: 14 - protein, 12 aa, Artificial Sequence
  artificial peptide composition
  MISC_FEATURE (8)..(8): Xaa at position 8 is 4-pyridyl alanine (4-Pal)
  MISC_FEATURE (12)..(12): Xaa at position 12 is D-tyrosine
DPEWWADXQKRX

SEQ ID NO: 15 - protein, 12 aa, Artificial Sequence
  artificial peptide composition
  MISC_FEATURE (1)..(1): Xaa at position 1 is D-arginine
  MISC_FEATURE (12)..(12): Xaa at position 12 is D-tyrosine
XPEWWMDYQKRX

SEQ ID NO: 16 - protein, 11 aa, Artificial Sequence
  artificial peptide composition
  MISC_FEATURE (1)..(1): Xaa at position 1 is proline or D-proline
  MISC_FEATURE (2)..(2): Xaa at position 2 is absent or glutamic acid
  MISC_FEATURE (7)..(7): Xaa at position 7 is tyrosine or phenylalanine
  MISC_FEATURE (11)..(11): Xaa at position 11 is tyrosine or D-tyrosine
XXWWMDXQKRX

SEQ ID NO: 17 - protein, 11 aa, Artificial Sequence
  artificial peptide composition
  MISC_FEATURE (11)..(11): Xaa at position 11 is D-tyrosine
PEWWMDYQKRX

SEQ ID NO: 18 - protein, 10 aa, Artificial Sequence
  artificial peptide composition
  MISC_FEATURE (10)..(10): Xaa at position 10 is D-tyrosine
EWWMDFQKRX

SEQ ID NO: 19 - protein, 11 aa, Artificial Sequence
  artificial peptide composition
  MISC_FEATURE (1)..(1): Xaa at position 1 is D-proline
  MISC_FEATURE (11)..(11): Xaa at position 11 is D-tyrosine
XEWWMDYQKRX

SEQ ID NO: 20 - protein, 15 aa, Artificial Sequence
  artificial peptide composition
  MISC_FEATURE (1)..(1): Xaa at position 1 is valine, D-valine, fluorinated D-valine, fluorinated D-alanine, or beta-D-alanine
  MISC_FEATURE (3)..(3): Xaa at position 3 is arginine, lysine, or N-methylated arginine
  MISC_FEATURE (5)..(5): Xaa at position 5 is glutamic acid or aspartic acid
  MISC_FEATURE (6)..(6): Xaa at position 6 is tryptophan or naphthylalanine (Nal)
  MISC_FEATURE (7)..(7): Xaa at position 7 is tryptophan, N-methylated tryptophan, or naphthylalanine (Nal)
  MISC_FEATURE (8)..(8): Xaa at position 8 is methionine or norleucine (Nle)
  MISC_FEATURE (9)..(9): Xaa at position 9 is aspartic acid or fluorinated glutamic acid
  MISC_FEATURE (10)..(10): Xaa at position 10 is tyrosine, threonine, or N-methylated tyrosine
  MISC_FEATURE (11)..(11): Xaa at position 11 is glutamine or asparagine
  MISC_FEATURE (12)..(12): Xaa at position 12 is lysine, arginine, or N-methylated lysine
  MISC_FEATURE (13)..(13): Xaa at position 13 is arginine, lysine, or N-methylated arginine
  MISC_FEATURE (14)..(14): Xaa at position 14 is tyrosine, threonine, or N-methylated tyrosine
  MISC_FEATURE (15)..(15): Xaa at position 15 is glycine or D-glycine
XGXPXXXXXXXXXXX

SEQ ID NO: 21 - protein, 15 aa, Bos taurus
VGRPEWWMDYQKRYG

SEQ ID NO: 22 - protein, 15 aa, Artificial Sequence
  artificial peptide composition
  MISC_FEATURE (8)..(8): Xaa at position 8 is norleucine
VGRPEWWXDYQKRYG

SEQ ID NO: 23 - protein, 15 aa, Artificial Sequence
  artificial peptide composition
  MISC_FEATURE (1)..(1): Xaa at position 1 is D-valine
  MISC_FEATURE (15)..(15): Xaa at position 15 is D-glycine
XGRPEWWMDYQKRYX

SEQ ID NO: 24 - protein, 15 aa, Artificial Sequence
  artificial peptide composition
  MISC_FEATURE (1)..(1): Xaa at position 1 is D-valine
  MISC_FEATURE (15)..(15): Xaa at position 15 is D-glycine
XGRPDWWMDYQKKYX

SEQ ID NO: 25 - protein, 15 aa, Artificial Sequence
  artificial peptide sequence
  MISC_FEATURE (1)..(1): Xaa at position 1 is D-valine
  MISC_FEATURE (15)..(15): Xaa at position 15 is D-glycine
XGRPDWWMDYQRRYX

SEQ ID NO: 26 - protein, 15 aa, Artificial Sequence
  artificial peptide composition
  MISC_FEATURE (1)..(1): Xaa at position 1 is D-valine
  MISC_FEATURE (15)..(15): Xaa at position 15 is D-glycine
XGRPDWWMDYQKRTX

SEQ ID NO: 27 - protein, 15 aa, Artificial Sequence
  artificial peptide composition
  MISC_FEATURE (1)..(1): Xaa at position 1 is D-valine
  MISC_FEATURE (15)..(15): Xaa at position 15 is D-glycine
XGKPDWWMDYQKRYX

SEQ ID NO: 28 - protein, 15 aa, Artificial Sequence
  artificial peptide composition
  MISC_FEATURE (1)..(1): Xaa at position 1 is D-valine
  MISC_FEATURE (15)..(15): Xaa at position 15 is D-glycine
XGRPDWWMDYNKRYX

SEQ ID NO: 29 - protein, 15 aa, Artificial Sequence
  artificial peptide composition
  MISC_FEATURE (1)..(1): Xaa at position 1 is D-valine
  MISC_FEATURE (15)..(15): Xaa at position 15 is D-glycine
XGRPDWWMDTQKRYX

SEQ ID NO: 30 - protein, 15 aa, Artificial Sequence
  artificial peptide composition
  MISC_FEATURE (15)..(15): Xaa at position 15 is D-glycine
VGRPDWWMDYQKRYX

SEQ ID NO: 31 - protein, 15 aa, Artificial Sequence
  artificial peptide composition
  MISC_FEATURE (1)..(1): Xaa at position 1 is D-valine
XGRPDWWMDYQKRYG

SEQ ID NO: 32 - protein, 15 aa, Artificial Sequence
  artificial peptide composition
VGRPDWWMDYQKRYG

SEQ ID NO: 33 - protein, 15 aa, Artificial Sequence
  artificial peptide sequence
  MISC_FEATURE (1)..(1): Xaa at position 1 is D-valine
  MISC_FEATURE (3)..(3): Xaa at position 3 is N-methylated arginine
  MISC_FEATURE (15)..(15): Xaa at position 15 is D-glycine
XGXPEWWMDYQKRYX

SEQ ID NO: 34 - protein, 15 aa, Artificial Sequence
  artificial peptide composition
  MISC_FEATURE (1)..(1): Xaa at position 1 is D-valine
  MISC_FEATURE (10)..(10): Xaa at position 10 is N-methylated tyrosine
  MISC_FEATURE (15)..(15): Xaa at position 15 is D-glycine
XGRPEWWMDXQKRYX

SEQ ID NO: 35 - protein, 15 aa, Artificial Sequence
  artificial peptide composition
  MISC_FEATURE (1)..(1): Xaa at position 1 is D-valine
  MISC_FEATURE (12)..(12): Xaa at position 12 is N-methylated lysine
  MISC_FEATURE (15)..(15): Xaa at position 15 is D-glycine
XGRPEWWMDYQXRYX

SEQ ID NO: 36 - protein, 15 aa, Artificial Sequence
  artificial peptide composition
  MISC_FEATURE (1)..(1): Xaa at position 1 is D-valine
  MISC_FEATURE (13)..(13): Xaa at position 13 is N-methylated arginine
  MISC_FEATURE (15)..(15): Xaa at position 15 is D-glycine
XGRPEWWMDYQKXYX

SEQ ID NO: 37 - protein, 15 aa, Artificial Sequence
  artificial peptide composition
  MISC_FEATURE (1)..(1): Xaa at position 1 is D-valine
  MISC_FEATURE (14)..(14): Xaa at position 14 is N-methylated tyrosine
  MISC_FEATURE (15)..(15): Xaa at position 15 is D-glycine
XGRPEWWMDYQKRXX

SEQ ID NO: 38 - protein, 15 aa, Artificial Sequence
  artificial peptide composition
  MISC_FEATURE (1)..(1): Xaa at position 1 is D-valine
  MISC_FEATURE (7)..(7): Xaa at position 7 is N-methylated tryptophan
  MISC_FEATURE (14)..(14): Xaa at position 14 is N-methylated tyrosine
  MISC_FEATURE (15)..(15): Xaa at position 15 is D-glycine
XGRPEWXMDYQKRXX

SEQ ID NO: 39 - protein, 15 aa, Artificial Sequence
  artificial peptide composition
  MISC_FEATURE (1)..(1): Xaa at position 1 is fluorinated D-valine
  MISC_FEATURE (15)..(15): Xaa at position 15 is D-glycine
XGRPEWWMDYQKRYX

SEQ ID NO: 40 - protein, 15 aa, Artificial Sequence
  artificial peptide composition
  MISC_FEATURE (1)..(1): Xaa at position 1 is fluorinated D-alanine
  MISC_FEATURE (15)..(15): Xaa at position 15 is D-glycine
XGRPEWWMDYQKRYX

SEQ ID NO: 41 - protein, 15 aa, Artificial Sequence
  artificial peptide composition
  MISC_FEATURE (1)..(1): Xaa at position 1 is D-valine
  MISC_FEATURE (9)..(9): Xaa at position 9 is fluorinated glutamic acid
  MISC_FEATURE (15)..(15): Xaa at position 15 is D-glycine
XGRPDWWMXYQKRYX

SEQ ID NO: 42 - protein, 15 aa, Artificial Sequence
  artificial peptide composition
  MISC_FEATURE (1)..(1): Xaa at position 1 is beta-D-alanine
  MISC_FEATURE (15)..(15): Xaa at position 15 is D-glycine
XGRPEWWMDYQKRYX

SEQ ID NO: 43 - protein, 15 aa, Artificial Sequence
  artificial peptide composition
  MISC_FEATURE (1)..(1): Xaa at position 1 is D-valine
  MISC_FEATURE (8)..(8): Xaa at position 8 is norleucine
  MISC_FEATURE (15)..(15): Xaa at position 15 is D-glycine
XGRPEWWXDYQKRYX

SEQ ID NO: 44 - protein, 15 aa, Artificial Sequence
  artificial peptide composition
  MISC_FEATURE (1)..(1): Xaa at position 1 is D-valine
  MISC_FEATURE (6)..(6): Xaa at position 6 is naphthylalanine (Nal)
  MISC_FEATURE (15)..(15): Xaa at position 15 is D-glycine
XGRPEXWMDYQKRYX

SEQ ID NO: 45 - protein, 15 aa, Artificial Sequence
  artificial peptide composition
  MISC_FEATURE (1)..(1): Xaa at position 1 is D-valine
  MISC_FEATURE (7)..(7): Xaa at position 7 is naphthylalanine (Nal)
  MISC_FEATURE (15)..(15): Xaa at position 15 is D-glycine
XGRPEWXMDYQKRYX

SEQ ID NO: 46 - protein, 12 aa, Artificial Sequence
  artificial peptide composition
  MISC_FEATURE (1)..(1): Xaa at position 1 is norarginine
  MISC_FEATURE (12)..(12): Xaa at position 12 is D-tyrosine
XPEWWMDYQKRX

SEQ ID NO: 47 - protein, 12 aa, Artificial Sequence
  artificial peptide composition
  MISC_FEATURE (1)..(1): Xaa at position 1 is norarginine
  MISC_FEATURE (12)..(12): Xaa at position 12 is D-tyrosine
XPEWWMDWQKRX

SEQ ID NO: 48 - protein, 9 aa, Artificial Sequence
  artificial peptide composition
EWWMDYQKR

SEQ ID NO: 49 - protein, 9 aa, Artificial Sequence
  artificial peptide composition
  MISC_FEATURE (9)..(9): Xaa at position 9 is D-tyrosine
WWMDYQKRX

SEQ ID NO: 50 - protein, 8 aa, Artificial Sequence
  artificial peptide composition
WWMDYQKR

SEQ ID NO: 51 - protein, 16 aa, Artificial Sequence
  artificial peptide composition
EVGRPEWWMDYQKRYG

SEQ ID NO: 52 - protein, 16 aa, Artificial Sequence
  artificial peptide composition
VGRPEWWMDYQKRYGK

SEQ ID NO: 53 - protein, 17 aa, Artificial Sequence
  artificial peptide composition
VGRPEWWMDYQKRYGKE

SEQ ID NO: 54 - protein, 15 aa, Artificial Sequence
  artificial peptide composition
VGRPEWWMDSQKRYG